European Patent Application EP 4 684 798 A2, published January 28, 2026. Title: A HIGH-CONCENTRATION COMPOSITION OF PD-1 ANTIBODY. Applicant: QILU PHARMACEUTICAL CO., LTD. The sequence listing filed with the application follows.

SEQUENCE LISTING (7 sequences)

SEQ ID NO: 1 - protein, 447 aa, Synthetic construct
QVQLVQSGVEVKKPGASVKVSCKASGYTFTNYYMYWVRQAPGQGLEWMGGINPSNGGTNFNEKFKNRVTLTTDSSTTTAYMELKSLQFDDTAVYYCARRDYRFDMGFDYWGQGTTVTVSSASTKGPSVFPLAPCSRSTSESTAALGCLVKDYFPEPVTVSWNSGALTSGVHTFPAVLQSSGLYSLSSVVTVPSSSLGTKTYTCNVDHKPSNTKVDKRVESKYGPPCPPCPAPEFLGGPSVFLFPPKPKDTLMISRTPEVTCVVVDVSQEDPEVQFNWYVDGVEVHNAKTKPREEQFNSTYRVVSVLTVLHQDWLNGKEYKCKVSNKGLPSSIEKTISKAKGQPREPQVYTLPPSQEEMTKNQVSLTCLVKGFYPSDIAVEWESNGQPENNYKTTPPVLDSDGSFFLYSRLTVDKSRWQEGNVFSCSVMHEALHNHYTQKSLSLSLGK

SEQ ID NO: 2 - protein, 218 aa, Synthetic construct
EIVLTQSPATLSLSPGERATLSCRASKGVSTSGYSYLHWYQQKPGQAPRLLIYLASYLESGVPARFSGSGSGTDFTLTISSLEPEDFAVYYCQHSRDLPLTFGGGTKVEIKRTVAAPSVFIFPPSDEQLKSGTASVVCLLNNFYPREAKVQWKVDNALQSGNSQESVTEQDSKDSTYSLSSTLTLSKADYEKHKVYACEVTHQGLSSPVTKSFNRGEC

SEQ ID NO: 3 - protein, 440 aa, Synthetic construct
GVEVKKPGASVKVSCKASGYTFTNYYMYWVRQAPGQGLEWMGGINPSNGGTNFNEKFKNRVTLTTDSSTTTAYMELKSLQFDDTAVYYCARRDYRFDMGFDYWGQGTTVTVSSASTKGPSVFPLAPCSRSTSESTAALGCLVKDYFPEPVTVSWNSGALTSGVHTFPAVLQSSGLYSLSSVVTVPSSSLGTKTYTCNVDHKPSNTKVDKRVESKYGPPCPPCPAPEFLGGPSVFLFPPKPKDTLMISRTPEVTCVVVDVSQEDPEVQFNWYVDGVEVHNAKTKPREEQFNSTYRVVSVLTVLHQDWLNGKEYKCKVSNKGLPSSIEKTISKAKGQPREPQVYTLPPSQEEMTKNQVSLTCLVKGFYPSDIAVEWESNGQPENNYKTTPPVLDSDGSFFLYSRLTVDKSRWQEGNVFSCSVMHEALHNHYTQKSLSLSLGK

SEQ ID NO: 4 - protein, 447 aa, Synthetic construct
QVQLVQSGVEVKKPGASVKVSCKASGYTFTNYYMYWVRQAPGQGLEWMGGINPSNGGTNFNEKFKNRVTLTTDSSTTTAYMELKSLQFDDTAVYYCARRDYRFDMGFDYWGQGTTVTVSSASTKGPSVFPLAPCSRSTSESTAALGCLVKDYFPEPVTVSWNSGALTSGVHTFPAVLQSSGLYSLSSVVTVPSSSLGTKTYTCNVDHKPSNTKVDKRVESKYGPPCPPCPAPEFLGGPSVFLFPPKPKDTLMISRTPEVTCVVVDVSQEDPEVQFNWYVDGVEVHNAKTKPREEQFNSTYRVVSVLTVLHQDWLNGKEYKCKVSNKGLPSSIEKTISKAKGQPREPQVCTLPPSQEEMTKNQVSLSCAVKGFYPSDIAVEWESNGQPENNYKTTPPVLDSDGSFFLVSRLTVDKSRWQEGNVFSCSVMHEALHNRFTQKSLSLSLGK

SEQ ID NO: 5 - protein, 440 aa, Synthetic construct
GVEVKKPGASVKVSCKASGYTFTNYYMYWVRQAPGQGLEWMGGINPSNGGTNFNEKFKNRVTLTTDSSTTTAYMELKSLQFDDTAVYYCARRDYRFDMGFDYWGQGTTVTVSSASTKGPSVFPLAPCSRSTSESTAALGCLVKDYFPEPVTVSWNSGALTSGVHTFPAVLQSSGLYSLSSVVTVPSSSLGTKTYTCNVDHKPSNTKVDKRVESKYGPPCPPCPAPEFLGGPSVFLFPPKPKDTLMISRTPEVTCVVVDVSQEDPEVQFNWYVDGVEVHNAKTKPREEQFNSTYRVVSVLTVLHQDWLNGKEYKCKVSNKGLPSSIEKTISKAKGQPREPQVYTLPPCQEEMTKNQVSLWCLVKGFYPSDIAVEWESNGQPENNYKTTPPVLDSDGSFFLYSRLTVDKSRWQEGNVFSCSVMHEALHNHYTQKSLSLSLGK

SEQ ID NO: 6 - protein, 5 aa, Synthetic construct
GVEVK

SEQ ID NO: 7 - protein, 12 aa, Synthetic construct
QVQLVQSGVEVK